European Patent Application EP 4 810 511 A1, published September 23, 2026. Title: Modified Fc-binding protein and method for producing thereof. Applicant: 東ソー株式会社. Application WO. The sequence listing filed with the application follows.

SEQUENCE LISTING (119 sequences)

SEQ ID NO: 1 - protein, 365 aa, Homo sapiens
  source 1..365: note = Human FcRn alpha chain
MGVPRPQPWALGLLLFLLPGSLGAESHLSLLYHLTAVSSPAPGTPAFWVSGWLGPQQYLSYNSLRGEAEPCGAWVWENQVSWYWEKETTDLRIKEKLFLEAFKALGGKGPYTLQGLLGCELGPDNTSVPTAKFALNGEEFMNFDLKQGTWGGDWPEALAISQRWQQQDKAANKELTFLLFSCPHRLREHLERGRGNLEWKEPPSMRLKARPSSPGFSVLTCSAFSFYPPELQLRFLRNGLAAGTGQGDFGPNSDGSFHASSSLTVKSGDEHHYCCIVQHAGLAQPLRVELESPAKSSVLVVGIVIGVLLLTAAAVGGALLWRRMRSGLPAPWISLRGDDTGVLLPTPGEAQDADLKDVNVIPATA

SEQ ID NO: 2 - protein, 119 aa, Homo sapiens
  source 1..119: note = beta2m(B2M)
MSRSVALAVLALLSLSGLEAIQRTPKIQVYSRHPAENGKSNFLNCYVSGFHPSDIEVDLLKNGERIEKVEHSDLSFSKDWSFYLLYYTEFTPTEKDEYACRVNHVTLSQPKIVKWDRDM

SEQ ID NO: 3 - protein, 26 aa, Escherichia coli
  source 1..26: note = MalE signal peptide
MKIKTGARILALSALTTMMFSASALA

SEQ ID NO: 4 - DNA, 35 bp, synthetic construct
  source 1..35: mol_type = other DNA; note = Oligonucleotide
tatacatatgaaaataaaaacaggtgcacgcatcc

SEQ ID NO: 5 - DNA, 39 bp, synthetic construct
  source 1..39: mol_type = other DNA; note = Oligonucleotide
gcattaacgacgatgatgttttccgcctcggctctcgcc

SEQ ID NO: 6 - DNA, 40 bp, synthetic construct
  source 1..40: mol_type = other DNA; note = Oligonucleotide
atcgtcgttaatgcggataatgcgaggatgcgtgcacctg

SEQ ID NO: 7 - DNA, 35 bp, synthetic construct
  source 1..35: mol_type = other DNA; note = Oligonucleotide
ttgtcccatggcttcttcgattttggcgagagccg

SEQ ID NO: 8 - DNA, 35 bp, synthetic construct; identical to SEQ ID NO: 4
  source 1..35: mol_type = other DNA; note = PCR forward primer

SEQ ID NO: 9 - DNA, 39 bp, synthetic construct; identical to SEQ ID NO: 5
  source 1..39: mol_type = other DNA; note = PCR reverse primer

SEQ ID NO: 10 - DNA, 23 bp, synthetic construct
  source 1..23: mol_type = other DNA; note = PCR forward primer
agtagtaggttgaggccgttgag

SEQ ID NO: 11 - DNA, 34 bp, synthetic construct
  source 1..34: mol_type = other DNA; note = PCR reverse primer
ttttcatatgtattatgtatatctccttcttaaa

SEQ ID NO: 12 - protein, 404 aa, synthetic construct
  source 1..404: note = FcRn(B2M-GS-EC_m7a)-6H
IQRTPKIQVYSRHPAENGKSNFLNCYVSGFHPSDIEVDLLKNGERIEKVEHSDLSFSKDWSFYLLYYTEFTPTEKDEYACRVNHVTLSQPKIVKWDRDMGGGGSGGGGSGGGGSGGGGSGGGGSAESHLSLLYHLTAVSSPAPGTPAFWVSGWLGPQQYLSYNSLRGEAEPRGAWVWEDQVSWYWEKETTDLRIKEKLFLEAFKALGGKGPYTLQGLLGCELGPDNTSVPTAKFALNGEEFMNFDLKQGTWDGDWPEALAISQRWQQQDKAANKELTFLLFSCPHRLREHLELGRGDLEWKEPPSMRLKARPSSPGFSVLTCSAFSFYPPELLLRFLRNGLAAGTGQGDFGPNSDGSFHASSSLTVKSGDEHHYCCIVQHAGLAQPLRVELESPAESSHHHHHH

SEQ ID NO: 13 - protein, 274 aa, synthetic construct
  source 1..274: note = EC_m7a
AESHLSLLYHLTAVSSPAPGTPAFWVSGWLGPQQYLSYNSLRGEAEPRGAWVWEDQVSWYWEKETTDLRIKEKLFLEAFKALGGKGPYTLQGLLGCELGPDNTSVPTAKFALNGEEFMNFDLKQGTWDGDWPEALAISQRWQQQDKAANKELTFLLFSCPHRLREHLELGRGDLEWKEPPSMRLKARPSSPGFSVLTCSAFSFYPPELLLRFLRNGLAAGTGQGDFGPNSDGSFHASSSLTVKSGDEHHYCCIVQHAGLAQPLRVELESPAESS

SEQ ID NO: 14 - DNA, 1212 bp, synthetic construct
  source 1..1212: mol_type = other DNA; note = FcRn(B2M-GS-EC_m7a)-6H DNA
attcaacgtacgccaaaaatccaagtttactctcgccatccggcagagaacggtaagtctaacttcctgaattgctacgtgtctggtttccacccgtccgacatcgaagttgacctcctcaaaaacggcgaacgtatcgaaaaagttgagcactctgacctcagcttcagcaaggactggtccttctacctgctctactacacggaattcaccccgaccgagaaggatgaatacgcctgccgtgttaatcacgttaccctgtctcagccgaaaattgtgaagtgggaccgcgatatgggtggtggtggctctggcggtggcggctctggcggtggcggttccggcggcggtggtagcggtggcggcggtagcgcggaaagccatctctccctgctgtatcatctgactgcggttagctctccggcaccaggtaccccagccttctgggtctctggttggctgggtccgcagcaatacctctcttataacagcctgcgcggtgaagcagaaccacgcggtgcgtgggtttgggaagaccaggtttcttggtactgggagaaagagacgaccgatctgcgcatcaaggaaaaactgttcctggaagccttcaaagcgctgggcggtaaaggtccatatactctccaaggcctgctgggctgtgaactcggtcctgacaacacctctgttccgacggccaaattcgcactgaacggtgaggagtttatgaattttgacctgaaacagggcacctgggatggcgattggccagaggcgctcgctatctcccaacgctggcagcagcaagataaggcagcgaacaaagaactgacgttcctcctgttttcttgcccgcaccgtctccgtgaacatctcgaacttggtcgtggtgacctcgaatggaaggagcctccgtctatgcgtctgaaagcgcgtccgtcttccccgggtttttctgtactcacttgttccgccttctccttttaccctccagaactcctgctgcgcttcctgcgcaatggcctcgctgcgggtacgggtcagggtgatttcggcccgaattctgacggctctttccacgcgtcttctagcctgacggtgaaatctggcgacgaacatcactactgctgcatcgtgcagcacgcgggtctcgcgcaaccgctccgcgttgagctcgaatcccctgccgaatcttctcatcatcatcatcatcat

SEQ ID NO: 15 - protein, 7 aa, synthetic construct
  source 1..7: note = Cystein tag
CRNDTCG

SEQ ID NO: 16 - DNA, 36 bp, synthetic construct
  source 1..36: mol_type = other DNA; note = PCR forward primer
gcctcggctctcgccattcaacgtacgccaaaaatc

SEQ ID NO: 17 - DNA, 69 bp, synthetic construct
  source 1..69: mol_type = other DNA; note = PCR reverse primer
agtgcggccgcaagcttatccgcaggtatcgttgcggcagtgatgatgatgatgatgagaggattcggc

SEQ ID NO: 18 - DNA, 42 bp, synthetic construct
  source 1..42: mol_type = other DNA; note = PCR forward primer
gcttgcggccgcactcgagcaccaccaccaccaccactgaga

SEQ ID NO: 19 - DNA, 36 bp, synthetic construct
  source 1..36: mol_type = other DNA; note = PCR reverse primer
ggcgagagccgaggcggaaaacatcatcgtcgttaa

SEQ ID NO: 20 - DNA, 19 bp, synthetic construct
  source 1..19: mol_type = other DNA; note = Sequence primer
ggatctcgacgctctccct

SEQ ID NO: 21 - DNA, 23 bp, synthetic construct
  source 1..23: mol_type = other DNA; note = Sequence primer
atgggcattcaacgtacgccaaa

SEQ ID NO: 22 - DNA, 24 bp, synthetic construct
  source 1..24: mol_type = other DNA; note = Sequence primer
ctgcgcatcaaggaaaaactgttc

SEQ ID NO: 23 - DNA, 20 bp, synthetic construct
  source 1..20: mol_type = other DNA; note = Sequence primer
cacgctggtctcgcgcaacc

SEQ ID NO: 24 - DNA, 21 bp, synthetic construct
  source 1..21: mol_type = other DNA; note = Sequence primer
atgctagttattgctcagcgg

SEQ ID NO: 25 - protein, 437 aa, synthetic construct
  source 1..437: note = MalE-FcRn(B2M-GS-EC_m7a)-6HC
MKIKTGARILALSALTTMMFSASALAIQRTPKIQVYSRHPAENGKSNFLNCYVSGFHPSDIEVDLLKNGERIEKVEHSDLSFSKDWSFYLLYYTEFTPTEKDEYACRVNHVTLSQPKIVKWDRDMGGGGSGGGGSGGGGSGGGGSGGGGSAESHLSLLYHLTAVSSPAPGTPAFWVSGWLGPQQYLSYNSLRGEAEPRGAWVWEDQVSWYWEKETTDLRIKEKLFLEAFKALGGKGPYTLQGLLGCELGPDNTSVPTAKFALNGEEFMNFDLKQGTWDGDWPEALAISQRWQQQDKAANKELTFLLFSCPHRLREHLELGRGDLEWKEPPSMRLKARPSSPGFSVLTCSAFSFYPPELLLRFLRNGLAAGTGQGDFGPNSDGSFHASSSLTVKSGDEHHYCCIVQHAGLAQPLRVELESPAESSHHHHHHCRNDTCG

SEQ ID NO: 26 - DNA, 1311 bp, synthetic construct
  source 1..1311: mol_type = other DNA; note = MalE-FcRn(B2M-GS-EC_m7a)-6HC DNA
atgaaaataaaaacaggtgcacgcatcctcgcattatccgcattaacgacgatgatgttttccgcctcggctctcgccattcaacgtacgccaaaaatccaagtatactcacgccatccggcagagaacggtaagtctaacttcctgaattgctacgtgtctggtttccacccgtccgacatcgaagttgacctcctcaaaaacggcgaacgtatcgaaaaagttgagcactctgacctcagcttcagcaaggactggtccttctacctgctctactacacggaattcaccccgaccgagaaggatgaatacgcctgccgtgttaatcacgttaccctgtctcagccgaaaattgtgaagtgggaccgcgatatgggtggtggtggctctggcggtggtggctctggcggtggcggttccggcggcggtggtagtggtggcggcggtagcgcggaaagccatctctccctgctgtatcatctgactgcggttagctctccggcaccaggtaccccagccttctgggtctctggttggctgggtccgcagcaatacctctcttataacagcctgcgcggtgaagcagaaccacgcggtgcgtgggtttgggaagaccaggtttcttggtactgggagaaagagacgaccgatctgcgcatcaaggaaaaactgttcctggaagccttcaaagcgctgggcggtaaaggtccatatactctccaaggcctgctgggctgtgaactcggtcctgacaacacctctgttccgacggccaaattcgcactgaacggtgaggagtttatgaattttgacctgaaacagggcacctgggatggcgattggccagaggcgctcgctatctcccaacgctggcagcagcaagataaggctgcgaacaaagaactgacgttcctcctgttttcttgcccgcaccgtctccgtgaacatctcgaacttggtcgtggtgacctcgaatggaaggagcctccgtctatgcgcctgaaagcgcgtccgtcttccccggggttttctgtactcacttgttccgccttctccttttaccctccagaactcctgctgcgcttcctgcgcaatggcctcgctgcgggtacgggtcagggtgatttcggcccgaattctgacggctctttccacgcgtcttctagcctgacggtgaaatctggcgacgaacatcactactgctgcatcgtgcagcacgctggtctcgcgcaaccgctccgcgttgagctcgaatcccctgccgaatcctctcatcatcatcatcatcactgccgcaacgatacctgcgga

SEQ ID NO: 27 - protein, 21 aa, Escherichia coli
  source 1..21: note = OmpA signal peptide
MKKTAIAIAVALAGFATVAQA

SEQ ID NO: 28 - protein, 432 aa, synthetic construct
  source 1..432: note = OmpA-FcRn(B2M-GS-EC_m7a)-6HC
MKKTAIAIAVALAGFATVAQAIQRTPKIQVYSRHPAENGKSNFLNCYVSGFHPSDIEVDLLKNGERIEKVEHSDLSFSKDWSFYLLYYTEFTPTEKDEYACRVNHVTLSQPKIVKWDRDMGGGGSGGGGSGGGGSGGGGSGGGGSAESHLSLLYHLTAVSSPAPGTPAFWVSGWLGPQQYLSYNSLRGEAEPRGAWVWEDQVSWYWEKETTDLRIKEKLFLEAFKALGGKGPYTLQGLLGCELGPDNTSVPTAKFALNGEEFMNFDLKQGTWDGDWPEALAISQRWQQQDKAANKELTFLLFSCPHRLREHLELGRGDLEWKEPPSMRLKARPSSPGFSVLTCSAFSFYPPELLLRFLRNGLAAGTGQGDFGPNSDGSFHASSSLTVKSGDEHHYCCIVQHAGLAQPLRVELESPAESSHHHHHHCRNDTCG

SEQ ID NO: 29 - DNA, 62 bp, synthetic construct
  source 1..62: mol_type = other DNA; note = PCR forward primer
gctggtttcgctaccgtagcgcaggccattcaacgtacgccaaaaatccaagtatactcacg

SEQ ID NO: 30 - DNA, 67 bp, synthetic construct
  source 1..67: mol_type = other DNA; note = PCR reverse primer
ggtagcgaaaccagccagtgccactgcaatcgcgatagctgtctttttcatatgtattatgtatatc

SEQ ID NO: 31 - DNA, 1296 bp, synthetic construct
  source 1..1296: mol_type = other DNA; note = OmpA-FcRn(B2M-GS-EC_m7a)-6HC DNA
atgaaaaagacagctatcgcgattgcagtggcactggctggtttcgctaccgtagcgcaggccattcaacgtacgccaaaaatccaagtatactcacgccatccggcagagaacggtaagtctaacttcctgaattgctacgtgtctggtttccacccgtccgacatcgaagttgacctcctcaaaaacggcgaacgtatcgaaaaagttgagcactctgacctcagcttcagcaaggactggtccttctacctgctctactacacggaattcaccccgaccgagaaggatgaatacgcctgccgtgttaatcacgttaccctgtctcagccgaaaattgtgaagtgggaccgcgatatgggtggtggtggctctggcggtggtggctctggcggtggcggttccggcggcggtggtagtggtggcggcggtagcgcggaaagccatctctccctgctgtatcatctgactgcggttagctctccggcaccaggtaccccagccttctgggtctctggttggctgggtccgcagcaatacctctcttataacagcctgcgcggtgaagcagaaccacgcggtgcgtgggtttgggaagaccaggtttcttggtactgggagaaagagacgaccgatctgcgcatcaaggaaaaactgttcctggaagccttcaaagcgctgggcggtaaaggtccatatactctccaaggcctgctgggctgtgaactcggtcctgacaacacctctgttccgacggccaaattcgcactgaacggtgaggagtttatgaattttgacctgaaacagggcacctgggatggcgattggccagaggcgctcgctatctcccaacgctggcagcagcaagataaggctgcgaacaaagaactgacgttcctcctgttttcttgcccgcaccgtctccgtgaacatctcgaacttggtcgtggtgacctcgaatggaaggagcctccgtctatgcgcctgaaagcgcgtccgtcttccccggggttttctgtactcacttgttccgccttctccttttaccctccagaactcctgctgcgcttcctgcgcaatggcctcgctgcgggtacgggtcagggtgatttcggcccgaattctgacggctctttccacgcgtcttctagcctgacggtgaaatctggcgacgaacatcactactgctgcatcgtgcagcacgctggtctcgcgcaaccgctccgcgttgagctcgaatcccctgccgaatcctctcatcatcatcatcatcactgccgcaacgatacctgcgga

SEQ ID NO: 32 - protein, 432 aa, synthetic construct
  source 1..432: note = Ca274A
MKKTAIAIAVALAGFATVAQAIQRTPKIQVYSRHPAENGKSNFLNCYVSGFHPSDIEVDLLKNGERIEKVEHSDLSFSKDWSFYLLYYTEFTPTEKDEYACRVNHVTLSQPKIVKWDRDMGGGGSGGGGSGGGGSGGGGSGGGGSAESHLSLLYHLTAVSSPAPGTPAFWVSGWLGPQQYLSYNSLRGEAEPRGAWVWEDQVSWYWEKETTDLRIKEKLFLEAFKALGGKGPYTLQGLLGCELGPDNTSVPTAKFALNGEEFMNFDLKQGTWDGDWPEALAISQRWQQQDKAANKELTFLLFSCPHRLREHLELGRGDLEWKEPPSMRLKARPSSPGFSVLTCSAFSFYPPELLLRFLRNGLAAGTGQGDFGPNSDGSFHASSSLTVKSGDEHHYACIVQHAGLAQPLRVELESPAESSHHHHHHCRNDTCG

SEQ ID NO: 33 - DNA, 25 bp, synthetic construct
  source 1..25: mol_type = other DNA; note = PCR forward primer for Ca274A
actacgcgtgcatcgtgcagcacgc

SEQ ID NO: 34 - DNA, 25 bp, synthetic construct
  source 1..25: mol_type = other DNA; note = PCR reverse primer for Ca274A
atgcacgcgtagtgatgttcgtcgc

SEQ ID NO: 35 - protein, 432 aa, synthetic construct
  source 1..432: note = Ca374D
MKKTAIAIAVALAGFATVAQAIQRTPKIQVYSRHPAENGKSNFLNCYVSGFHPSDIEVDLLKNGERIEKVEHSDLSFSKDWSFYLLYYTEFTPTEKDEYACRVNHVTLSQPKIVKWDRDMGGGGSGGGGSGGGGSGGGGSGGGGSAESHLSLLYHLTAVSSPAPGTPAFWVSGWLGPQQYLSYNSLRGEAEPRGAWVWEDQVSWYWEKETTDLRIKEKLFLEAFKALGGKGPYTLQGLLGCELGPDNTSVPTAKFALNGEEFMNFDLKQGTWDGDWPEALAISQRWQQQDKAANKELTFLLFSCPHRLREHLELGRGDLEWKEPPSMRLKARPSSPGFSVLTCSAFSFYPPELLLRFLRNGLAAGTGQGDFGPNSDGSFHASSSLTVKSGDEHHYDCIVQHAGLAQPLRVELESPAESSHHHHHHCRNDTCG

SEQ ID NO: 36 - DNA, 25 bp, synthetic construct
  source 1..25: mol_type = other DNA; note = PCR forward primer for Ca374D
actacgattgcatcgtgcagcacgc

SEQ ID NO: 37 - DNA, 25 bp, synthetic construct
  source 1..25: mol_type = other DNA; note = PCR reverse primer for Ca374D
atgcaatcgtagtgatgttcgtcgc

SEQ ID NO: 38 - protein, 432 aa, synthetic construct
  source 1..432: note = Ca374E
MKKTAIAIAVALAGFATVAQAIQRTPKIQVYSRHPAENGKSNFLNCYVSGFHPSDIEVDLLKNGERIEKVEHSDLSFSKDWSFYLLYYTEFTPTEKDEYACRVNHVTLSQPKIVKWDRDMGGGGSGGGGSGGGGSGGGGSGGGGSAESHLSLLYHLTAVSSPAPGTPAFWVSGWLGPQQYLSYNSLRGEAEPRGAWVWEDQVSWYWEKETTDLRIKEKLFLEAFKALGGKGPYTLQGLLGCELGPDNTSVPTAKFALNGEEFMNFDLKQGTWDGDWPEALAISQRWQQQDKAANKELTFLLFSCPHRLREHLELGRGDLEWKEPPSMRLKARPSSPGFSVLTCSAFSFYPPELLLRFLRNGLAAGTGQGDFGPNSDGSFHASSSLTVKSGDEHHYECIVQHAGLAQPLRVELESPAESSHHHHHHCRNDTCG

SEQ ID NO: 39 - DNA, 25 bp, synthetic construct
  source 1..25: mol_type = other DNA; note = PCR forward primer for Ca274E
actacgaatgcatcgtgcagcacgc

SEQ ID NO: 40 - DNA, 25 bp, synthetic construct
  source 1..25: mol_type = other DNA; note = PCR reverse primer for Ca274E
atgcattcgtagtgatgttcgtcgc

SEQ ID NO: 41 - protein, 432 aa, synthetic construct
  source 1..432: note = Ca274F
MKKTAIAIAVALAGFATVAQAIQRTPKIQVYSRHPAENGKSNFLNCYVSGFHPSDIEVDLLKNGERIEKVEHSDLSFSKDWSFYLLYYTEFTPTEKDEYACRVNHVTLSQPKIVKWDRDMGGGGSGGGGSGGGGSGGGGSGGGGSAESHLSLLYHLTAVSSPAPGTPAFWVSGWLGPQQYLSYNSLRGEAEPRGAWVWEDQVSWYWEKETTDLRIKEKLFLEAFKALGGKGPYTLQGLLGCELGPDNTSVPTAKFALNGEEFMNFDLKQGTWDGDWPEALAISQRWQQQDKAANKELTFLLFSCPHRLREHLELGRGDLEWKEPPSMRLKARPSSPGFSVLTCSAFSFYPPELLLRFLRNGLAAGTGQGDFGPNSDGSFHASSSLTVKSGDEHHYFCIVQHAGLAQPLRVELESPAESSHHHHHHCRNDTCG

SEQ ID NO: 42 - DNA, 25 bp, synthetic construct
  source 1..25: mol_type = other DNA; note = PCR forward primer for Ca274F
actacttttgcatcgtgcagcacgc

SEQ ID NO: 43 - DNA, 25 bp, synthetic construct
  source 1..25: mol_type = other DNA; note = PCR reverse primer for Ca274F
atgcaaaagtagtgatgttcgtcgc

SEQ ID NO: 44 - protein, 432 aa, synthetic construct
  source 1..432: note = Ca274G
MKKTAIAIAVALAGFATVAQAIQRTPKIQVYSRHPAENGKSNFLNCYVSGFHPSDIEVDLLKNGERIEKVEHSDLSFSKDWSFYLLYYTEFTPTEKDEYACRVNHVTLSQPKIVKWDRDMGGGGSGGGGSGGGGSGGGGSGGGGSAESHLSLLYHLTAVSSPAPGTPAFWVSGWLGPQQYLSYNSLRGEAEPRGAWVWEDQVSWYWEKETTDLRIKEKLFLEAFKALGGKGPYTLQGLLGCELGPDNTSVPTAKFALNGEEFMNFDLKQGTWDGDWPEALAISQRWQQQDKAANKELTFLLFSCPHRLREHLELGRGDLEWKEPPSMRLKARPSSPGFSVLTCSAFSFYPPELLLRFLRNGLAAGTGQGDFGPNSDGSFHASSSLTVKSGDEHHYGCIVQHAGLAQPLRVELESPAESSHHHHHHCRNDTCG

SEQ ID NO: 45 - DNA, 25 bp, synthetic construct
  source 1..25: mol_type = other DNA; note = PCR forward primer for Ca274G
actacggctgcatcgtgcagcacgc

SEQ ID NO: 46 - DNA, 25 bp, synthetic construct
  source 1..25: mol_type = other DNA; note = PCR reverse primer for Ca274G
atgcagccgtagtgatgttcgtcgc

SEQ ID NO: 47 - protein, 432 aa, synthetic construct
  source 1..432: note = Ca274H
MKKTAIAIAVALAGFATVAQAIQRTPKIQVYSRHPAENGKSNFLNCYVSGFHPSDIEVDLLKNGERIEKVEHSDLSFSKDWSFYLLYYTEFTPTEKDEYACRVNHVTLSQPKIVKWDRDMGGGGSGGGGSGGGGSGGGGSGGGGSAESHLSLLYHLTAVSSPAPGTPAFWVSGWLGPQQYLSYNSLRGEAEPRGAWVWEDQVSWYWEKETTDLRIKEKLFLEAFKALGGKGPYTLQGLLGCELGPDNTSVPTAKFALNGEEFMNFDLKQGTWDGDWPEALAISQRWQQQDKAANKELTFLLFSCPHRLREHLELGRGDLEWKEPPSMRLKARPSSPGFSVLTCSAFSFYPPELLLRFLRNGLAAGTGQGDFGPNSDGSFHASSSLTVKSGDEHHYHCIVQHAGLAQPLRVELESPAESSHHHHHHCRNDTCG

SEQ ID NO: 48 - DNA, 25 bp, synthetic construct
  source 1..25: mol_type = other DNA; note = PCR forward primer for Ca274H
actaccattgcatcgtgcagcacgc

SEQ ID NO: 49 - DNA, 25 bp, synthetic construct
  source 1..25: mol_type = other DNA; note = PCR reverse primer for Ca274H
atgcaatggtagtgatgttcgtcgc

SEQ ID NO: 50 - protein, 432 aa, synthetic construct
  source 1..432: note = Ca274I
MKKTAIAIAVALAGFATVAQAIQRTPKIQVYSRHPAENGKSNFLNCYVSGFHPSDIEVDLLKNGERIEKVEHSDLSFSKDWSFYLLYYTEFTPTEKDEYACRVNHVTLSQPKIVKWDRDMGGGGSGGGGSGGGGSGGGGSGGGGSAESHLSLLYHLTAVSSPAPGTPAFWVSGWLGPQQYLSYNSLRGEAEPRGAWVWEDQVSWYWEKETTDLRIKEKLFLEAFKALGGKGPYTLQGLLGCELGPDNTSVPTAKFALNGEEFMNFDLKQGTWDGDWPEALAISQRWQQQDKAANKELTFLLFSCPHRLREHLELGRGDLEWKEPPSMRLKARPSSPGFSVLTCSAFSFYPPELLLRFLRNGLAAGTGQGDFGPNSDGSFHASSSLTVKSGDEHHYICIVQHAGLAQPLRVELESPAESSHHHHHHCRNDTCG

SEQ ID NO: 51 - DNA, 25 bp, synthetic construct
  source 1..25: mol_type = other DNA; note = PCR forward primer for Ca274I
actacatttgcatcgtgcagcacgc

SEQ ID NO: 52 - DNA, 25 bp, synthetic construct
  source 1..25: mol_type = other DNA; note = PCR reverse primerfor Ca274I
atgcaaatgtagtgatgttcgtcgc

SEQ ID NO: 53 - protein, 432 aa, synthetic construct
  source 1..432: note = Ca274K
MKKTAIAIAVALAGFATVAQAIQRTPKIQVYSRHPAENGKSNFLNCYVSGFHPSDIEVDLLKNGERIEKVEHSDLSFSKDWSFYLLYYTEFTPTEKDEYACRVNHVTLSQPKIVKWDRDMGGGGSGGGGSGGGGSGGGGSGGGGSAESHLSLLYHLTAVSSPAPGTPAFWVSGWLGPQQYLSYNSLRGEAEPRGAWVWEDQVSWYWEKETTDLRIKEKLFLEAFKALGGKGPYTLQGLLGCELGPDNTSVPTAKFALNGEEFMNFDLKQGTWDGDWPEALAISQRWQQQDKAANKELTFLLFSCPHRLREHLELGRGDLEWKEPPSMRLKARPSSPGFSVLTCSAFSFYPPELLLRFLRNGLAAGTGQGDFGPNSDGSFHASSSLTVKSGDEHHYKCIVQHAGLAQPLRVELESPAESSHHHHHHCRNDTCG

SEQ ID NO: 54 - DNA, 25 bp, synthetic construct
  source 1..25: mol_type = other DNA; note = PCR forward primer for Ca274K
actacaaatgcatcgtgcagcacgc

SEQ ID NO: 55 - DNA, 25 bp, synthetic construct
  source 1..25: mol_type = other DNA; note = PCR reverse primer for Ca274K
atgcatttgtagtgatgttcgtcgc

SEQ ID NO: 56 - protein, 432 aa, synthetic construct
  source 1..432: note = Ca274L
MKKTAIAIAVALAGFATVAQAIQRTPKIQVYSRHPAENGKSNFLNCYVSGFHPSDIEVDLLKNGERIEKVEHSDLSFSKDWSFYLLYYTEFTPTEKDEYACRVNHVTLSQPKIVKWDRDMGGGGSGGGGSGGGGSGGGGSGGGGSAESHLSLLYHLTAVSSPAPGTPAFWVSGWLGPQQYLSYNSLRGEAEPRGAWVWEDQVSWYWEKETTDLRIKEKLFLEAFKALGGKGPYTLQGLLGCELGPDNTSVPTAKFALNGEEFMNFDLKQGTWDGDWPEALAISQRWQQQDKAANKELTFLLFSCPHRLREHLELGRGDLEWKEPPSMRLKARPSSPGFSVLTCSAFSFYPPELLLRFLRNGLAAGTGQGDFGPNSDGSFHASSSLTVKSGDEHHYLCIVQHAGLAQPLRVELESPAESSHHHHHHCRNDTCG

SEQ ID NO: 57 - DNA, 25 bp, synthetic construct
  source 1..25: mol_type = other DNA; note = PCR forward primer for Ca274L
actacctgtgcatcgtgcagcacgc

SEQ ID NO: 58 - DNA, 25 bp, synthetic construct
  source 1..25: mol_type = other DNA; note = PCR reverse primer for Ca274L
atgcacaggtagtgatgttcgtcgc

SEQ ID NO: 59 - protein, 432 aa, synthetic construct
  source 1..432: note = Ca274M
MKKTAIAIAVALAGFATVAQAIQRTPKIQVYSRHPAENGKSNFLNCYVSGFHPSDIEVDLLKNGERIEKVEHSDLSFSKDWSFYLLYYTEFTPTEKDEYACRVNHVTLSQPKIVKWDRDMGGGGSGGGGSGGGGSGGGGSGGGGSAESHLSLLYHLTAVSSPAPGTPAFWVSGWLGPQQYLSYNSLRGEAEPRGAWVWEDQVSWYWEKETTDLRIKEKLFLEAFKALGGKGPYTLQGLLGCELGPDNTSVPTAKFALNGEEFMNFDLKQGTWDGDWPEALAISQRWQQQDKAANKELTFLLFSCPHRLREHLELGRGDLEWKEPPSMRLKARPSSPGFSVLTCSAFSFYPPELLLRFLRNGLAAGTGQGDFGPNSDGSFHASSSLTVKSGDEHHYMCIVQHAGLAQPLRVELESPAESSHHHHHHCRNDTCG

SEQ ID NO: 60 - DNA, 25 bp, synthetic construct
  source 1..25: mol_type = other DNA; note = PCR forward primer forCa274M
actacatgtgcatcgtgcagcacgc

SEQ ID NO: 61 - DNA, 25 bp, synthetic construct
  source 1..25: mol_type = other DNA; note = PCR reverse primer for Ca274M
atgcacatgtagtgatgttcgtcgc

SEQ ID NO: 62 - protein, 432 aa, synthetic construct
  source 1..432: note = Ca274N
MKKTAIAIAVALAGFATVAQAIQRTPKIQVYSRHPAENGKSNFLNCYVSGFHPSDIEVDLLKNGERIEKVEHSDLSFSKDWSFYLLYYTEFTPTEKDEYACRVNHVTLSQPKIVKWDRDMGGGGSGGGGSGGGGSGGGGSGGGGSAESHLSLLYHLTAVSSPAPGTPAFWVSGWLGPQQYLSYNSLRGEAEPRGAWVWEDQVSWYWEKETTDLRIKEKLFLEAFKALGGKGPYTLQGLLGCELGPDNTSVPTAKFALNGEEFMNFDLKQGTWDGDWPEALAISQRWQQQDKAANKELTFLLFSCPHRLREHLELGRGDLEWKEPPSMRLKARPSSPGFSVLTCSAFSFYPPELLLRFLRNGLAAGTGQGDFGPNSDGSFHASSSLTVKSGDEHHYNCIVQHAGLAQPLRVELESPAESSHHHHHHCRNDTCG

SEQ ID NO: 63 - DNA, 25 bp, synthetic construct
  source 1..25: mol_type = other DNA; note = PCR forward primer for Ca274N
actacaattgcatcgtgcagcacgc

SEQ ID NO: 64 - DNA, 25 bp, synthetic construct
  source 1..25: mol_type = other DNA; note = PCR reverse primer for Ca274N
atgcaattgtagtgatgttcgtcgc

SEQ ID NO: 65 - protein, 432 aa, synthetic construct
  source 1..432: note = Ca274P
MKKTAIAIAVALAGFATVAQAIQRTPKIQVYSRHPAENGKSNFLNCYVSGFHPSDIEVDLLKNGERIEKVEHSDLSFSKDWSFYLLYYTEFTPTEKDEYACRVNHVTLSQPKIVKWDRDMGGGGSGGGGSGGGGSGGGGSGGGGSAESHLSLLYHLTAVSSPAPGTPAFWVSGWLGPQQYLSYNSLRGEAEPRGAWVWEDQVSWYWEKETTDLRIKEKLFLEAFKALGGKGPYTLQGLLGCELGPDNTSVPTAKFALNGEEFMNFDLKQGTWDGDWPEALAISQRWQQQDKAANKELTFLLFSCPHRLREHLELGRGDLEWKEPPSMRLKARPSSPGFSVLTCSAFSFYPPELLLRFLRNGLAAGTGQGDFGPNSDGSFHASSSLTVKSGDEHHYPCIVQHAGLAQPLRVELESPAESSHHHHHHCRNDTCG

SEQ ID NO: 66 - DNA, 25 bp, synthetic construct
  source 1..25: mol_type = other DNA; note = PCR forward primer for Ca274P
actacccgtgcatcgtgcagcacgc

SEQ ID NO: 67 - DNA, 25 bp, synthetic construct
  source 1..25: mol_type = other DNA; note = PCR reverse primer for Ca274P
atgcacgggtagtgatgttcgtcgc

SEQ ID NO: 68 - protein, 432 aa, synthetic construct
  source 1..432: note = Ca274Q
MKKTAIAIAVALAGFATVAQAIQRTPKIQVYSRHPAENGKSNFLNCYVSGFHPSDIEVDLLKNGERIEKVEHSDLSFSKDWSFYLLYYTEFTPTEKDEYACRVNHVTLSQPKIVKWDRDMGGGGSGGGGSGGGGSGGGGSGGGGSAESHLSLLYHLTAVSSPAPGTPAFWVSGWLGPQQYLSYNSLRGEAEPRGAWVWEDQVSWYWEKETTDLRIKEKLFLEAFKALGGKGPYTLQGLLGCELGPDNTSVPTAKFALNGEEFMNFDLKQGTWDGDWPEALAISQRWQQQDKAANKELTFLLFSCPHRLREHLELGRGDLEWKEPPSMRLKARPSSPGFSVLTCSAFSFYPPELLLRFLRNGLAAGTGQGDFGPNSDGSFHASSSLTVKSGDEHHYQCIVQHAGLAQPLRVELESPAESSHHHHHHCRNDTCG

SEQ ID NO: 69 - DNA, 25 bp, synthetic construct
  source 1..25: mol_type = other DNA; note = PCR forward primer for Ca274Q
actaccagtgcatcgtgcagcacgc

SEQ ID NO: 70 - DNA, 25 bp, synthetic construct
  source 1..25: mol_type = other DNA; note = PCR reverse primer for Ca274Q
atgcactggtagtgatgttcgtcgc

SEQ ID NO: 71 - protein, 432 aa, synthetic construct
  source 1..432: note = Ca274R
MKKTAIAIAVALAGFATVAQAIQRTPKIQVYSRHPAENGKSNFLNCYVSGFHPSDIEVDLLKNGERIEKVEHSDLSFSKDWSFYLLYYTEFTPTEKDEYACRVNHVTLSQPKIVKWDRDMGGGGSGGGGSGGGGSGGGGSGGGGSAESHLSLLYHLTAVSSPAPGTPAFWVSGWLGPQQYLSYNSLRGEAEPRGAWVWEDQVSWYWEKETTDLRIKEKLFLEAFKALGGKGPYTLQGLLGCELGPDNTSVPTAKFALNGEEFMNFDLKQGTWDGDWPEALAISQRWQQQDKAANKELTFLLFSCPHRLREHLELGRGDLEWKEPPSMRLKARPSSPGFSVLTCSAFSFYPPELLLRFLRNGLAAGTGQGDFGPNSDGSFHASSSLTVKSGDEHHYRCIVQHAGLAQPLRVELESPAESSHHHHHHCRNDTCG

SEQ ID NO: 72 - DNA, 25 bp, synthetic construct
  source 1..25: mol_type = other DNA; note = PCR forward primer for Ca274R
actaccgctgcatcgtgcagcacgc

SEQ ID NO: 73 - DNA, 25 bp, synthetic construct
  source 1..25: mol_type = other DNA; note = PCR reverse primer for Ca274R
atgcagcggtagtgatgttcgtcgc

SEQ ID NO: 74 - protein, 432 aa, synthetic construct
  source 1..432: note = Ca274S
MKKTAIAIAVALAGFATVAQAIQRTPKIQVYSRHPAENGKSNFLNCYVSGFHPSDIEVDLLKNGERIEKVEHSDLSFSKDWSFYLLYYTEFTPTEKDEYACRVNHVTLSQPKIVKWDRDMGGGGSGGGGSGGGGSGGGGSGGGGSAESHLSLLYHLTAVSSPAPGTPAFWVSGWLGPQQYLSYNSLRGEAEPRGAWVWEDQVSWYWEKETTDLRIKEKLFLEAFKALGGKGPYTLQGLLGCELGPDNTSVPTAKFALNGEEFMNFDLKQGTWDGDWPEALAISQRWQQQDKAANKELTFLLFSCPHRLREHLELGRGDLEWKEPPSMRLKARPSSPGFSVLTCSAFSFYPPELLLRFLRNGLAAGTGQGDFGPNSDGSFHASSSLTVKSGDEHHYSCIVQHAGLAQPLRVELESPAESSHHHHHHCRNDTCG

SEQ ID NO: 75 - DNA, 25 bp, synthetic construct
  source 1..25: mol_type = other DNA; note = PCR forward primer for Ca274S
actacagctgcatcgtgcagcacgc

SEQ ID NO: 76 - DNA, 25 bp, synthetic construct
  source 1..25: mol_type = other DNA; note = PCR reverse primer for Ca274S
atgcagctgtagtgatgttcgtcgc

SEQ ID NO: 77 - protein, 432 aa, synthetic construct
  source 1..432: note = Ca274T
MKKTAIAIAVALAGFATVAQAIQRTPKIQVYSRHPAENGKSNFLNCYVSGFHPSDIEVDLLKNGERIEKVEHSDLSFSKDWSFYLLYYTEFTPTEKDEYACRVNHVTLSQPKIVKWDRDMGGGGSGGGGSGGGGSGGGGSGGGGSAESHLSLLYHLTAVSSPAPGTPAFWVSGWLGPQQYLSYNSLRGEAEPRGAWVWEDQVSWYWEKETTDLRIKEKLFLEAFKALGGKGPYTLQGLLGCELGPDNTSVPTAKFALNGEEFMNFDLKQGTWDGDWPEALAISQRWQQQDKAANKELTFLLFSCPHRLREHLELGRGDLEWKEPPSMRLKARPSSPGFSVLTCSAFSFYPPELLLRFLRNGLAAGTGQGDFGPNSDGSFHASSSLTVKSGDEHHYTCIVQHAGLAQPLRVELESPAESSHHHHHHCRNDTCG

SEQ ID NO: 78 - DNA, 25 bp, synthetic construct
  source 1..25: mol_type = other DNA; note = PCR forward primer for Ca274T
actacacctgcatcgtgcagcacgc

SEQ ID NO: 79 - DNA, 25 bp, synthetic construct
  source 1..25: mol_type = other DNA; note = PCR reverse primer for Ca274T
atgcaggtgtagtgatgttcgtcgc

SEQ ID NO: 80 - protein, 432 aa, synthetic construct
  source 1..432: note = Ca274V
MKKTAIAIAVALAGFATVAQAIQRTPKIQVYSRHPAENGKSNFLNCYVSGFHPSDIEVDLLKNGERIEKVEHSDLSFSKDWSFYLLYYTEFTPTEKDEYACRVNHVTLSQPKIVKWDRDMGGGGSGGGGSGGGGSGGGGSGGGGSAESHLSLLYHLTAVSSPAPGTPAFWVSGWLGPQQYLSYNSLRGEAEPRGAWVWEDQVSWYWEKETTDLRIKEKLFLEAFKALGGKGPYTLQGLLGCELGPDNTSVPTAKFALNGEEFMNFDLKQGTWDGDWPEALAISQRWQQQDKAANKELTFLLFSCPHRLREHLELGRGDLEWKEPPSMRLKARPSSPGFSVLTCSAFSFYPPELLLRFLRNGLAAGTGQGDFGPNSDGSFHASSSLTVKSGDEHHYVCIVQHAGLAQPLRVELESPAESSHHHHHHCRNDTCG

SEQ ID NO: 81 - DNA, 25 bp, synthetic construct
  source 1..25: mol_type = other DNA; note = PCR forward primer for Ca274V
actacgtgtgcatcgtgcagcacgc

SEQ ID NO: 82 - DNA, 25 bp, synthetic construct
  source 1..25: mol_type = other DNA; note = PCR reverse primer for Ca274V
atgcacacgtagtgatgttcgtcgc

SEQ ID NO: 83 - protein, 432 aa, synthetic construct
  source 1..432: note = Ca274W
MKKTAIAIAVALAGFATVAQAIQRTPKIQVYSRHPAENGKSNFLNCYVSGFHPSDIEVDLLKNGERIEKVEHSDLSFSKDWSFYLLYYTEFTPTEKDEYACRVNHVTLSQPKIVKWDRDMGGGGSGGGGSGGGGSGGGGSGGGGSAESHLSLLYHLTAVSSPAPGTPAFWVSGWLGPQQYLSYNSLRGEAEPRGAWVWEDQVSWYWEKETTDLRIKEKLFLEAFKALGGKGPYTLQGLLGCELGPDNTSVPTAKFALNGEEFMNFDLKQGTWDGDWPEALAISQRWQQQDKAANKELTFLLFSCPHRLREHLELGRGDLEWKEPPSMRLKARPSSPGFSVLTCSAFSFYPPELLLRFLRNGLAAGTGQGDFGPNSDGSFHASSSLTVKSGDEHHYWCIVQHAGLAQPLRVELESPAESSHHHHHHCRNDTCG

SEQ ID NO: 84 - DNA, 25 bp, synthetic construct
  source 1..25: mol_type = other DNA; note = PCR forward primer for Ca274W
actactggtgcatcgtgcagcacgc

SEQ ID NO: 85 - DNA, 25 bp, synthetic construct
  source 1..25: mol_type = other DNA; note = PCR reverse primer for Ca274W
atgcaccagtagtgatgttcgtcgc

SEQ ID NO: 86 - protein, 432 aa, synthetic construct
  source 1..432: note = Ca274Y
MKKTAIAIAVALAGFATVAQAIQRTPKIQVYSRHPAENGKSNFLNCYVSGFHPSDIEVDLLKNGERIEKVEHSDLSFSKDWSFYLLYYTEFTPTEKDEYACRVNHVTLSQPKIVKWDRDMGGGGSGGGGSGGGGSGGGGSGGGGSAESHLSLLYHLTAVSSPAPGTPAFWVSGWLGPQQYLSYNSLRGEAEPRGAWVWEDQVSWYWEKETTDLRIKEKLFLEAFKALGGKGPYTLQGLLGCELGPDNTSVPTAKFALNGEEFMNFDLKQGTWDGDWPEALAISQRWQQQDKAANKELTFLLFSCPHRLREHLELGRGDLEWKEPPSMRLKARPSSPGFSVLTCSAFSFYPPELLLRFLRNGLAAGTGQGDFGPNSDGSFHASSSLTVKSGDEHHYYCIVQHAGLAQPLRVELESPAESSHHHHHHCRNDTCG

SEQ ID NO: 87 - DNA, 25 bp, synthetic construct
  source 1..25: mol_type = other DNA; note = PCR forward primer for Ca274Y
actactattgcatcgtgcagcacgc

SEQ ID NO: 88 - DNA, 25 bp, synthetic construct
  source 1..25: mol_type = other DNA; note = PCR reverse primer for Ca274Y
atgcaatagtagtgatgttcgtcgc

SEQ ID NO: 89 - protein, 432 aa, synthetic construct
  source 1..432: note = OmpA-FcRn(B2M-GS-EC_m6)-6HC
MKKTAIAIAVALAGFATVAQAIQRTPKIQVYSRHPAENGKSNFLNCYVSGFHPSDIEVDLLKNGERIEKVEHSDLSFSKDWSFYLLYYTEFTPTEKDEYACRVNHVTLSQPKIVKWDRDMGGGGSGGGGSGGGGSGGGGSGGGGSAESHLSLLYHLTAVSSPAPGTPAFWVSGWLGPQQYLSYNSLRGEAEPRGAWVWEDQVSWYWEKETTDLRIKEKLFLEAFKALGGKGPYTLQGLLGCELGPDNTSVPTAKFALNGEEFMNFDLKQGTWGGDWPEALAISQRWQQQDKAANKELTFLLFSCPHRLREHLELGRGDLEWKEPPSMRLKARPSSPGFSVLTCSAFSFYPPELLLRFLRNGLAAGTGQGDFGPNSDGSFHASSSLTVKSGDEHHYCCIVQHAGLAQPLRVELESPAESSHHHHHHCRNDTCG

SEQ ID NO: 90 - DNA, 25 bp, synthetic construct
  source 1..25: mol_type = other DNA; note = PCR forward primer for EC_m6
cctggggcggcgattggccagaggc

SEQ ID NO: 91 - DNA, 25 bp, synthetic construct
  source 1..25: mol_type = other DNA; note = PCR reverse primer for EC_m6
tcgccgccccaggtgccctgtttca

SEQ ID NO: 92 - protein, 432 aa, synthetic construct
  source 1..432: note = OmpA-FcRn(B2M-GS-EC_m7b)-6HC
MKKTAIAIAVALAGFATVAQAIQRTPKIQVYSRHPAENGKSNFLNCYVSGFHPSDIEVDLLKNGERIEKVEHSDLSFSKDWSFYLLYYTEFTPTEKDEYACRVNHVTLSQPKIVKWDRDMGGGGSGGGGSGGGGSGGGGSGGGGSAESHLSLLYHLTAVSSPAPGTPAFWVSGWLGPQQYLSYNSLRGEAEPRGAWVWEDQVSWYWEKETTDLRIKEKLFLEAFKALGGKGPYTLQGLLGCELGPDNTSVPTAKFALNGEEFMNFDLKQGTWGGDWPEALAISQRWQQQDKAANKELTFLLFSCPHRLREHLELGRGDLEWKEPPSMRLKARPSSPGFSVLTCSAFSFYPPELLLRFLRNGLAAGTGQGDFGPNSDGSFHASSSLTVKSGDEHHYSCIVQHAGLAQPLRVELESPAESSHHHHHHCRNDTCG

SEQ ID NO: 93 - protein, 432 aa, synthetic construct
  source 1..432: note = OmpA-FcRn(B2M-GS-EC_m10)-6HC
MKKTAIAIAVALAGFATVAQAIQRTPKIQVYSRHPAENGKSNFLNCYVSGFHPSDIEVDLLKNGERIEKVEHSDLSFSKDWSFYLLYYTEFTPTEKDEYACRVNHVTLSQPKIVKWDRDMGGGGSGGGGSGGGGSGGGGSGGGGSAESHLSLLYHLTAVSSPAPGTPAFWVSGWLGPQQYLSYNSLRGEAEPRGAWVWEDQDSWYWEKETTDLRIKEELFLEAFKALGGKGPYTLQGLLGCELGPDNTSVPTAKFALNGEEFMNFDLKQGTWGGDWPEALAISQRWQQQDKAADKELTFLLFSCPHRLREHLELGRGDLEWKEPPSMRLKARPSSPGFSVLTCSAFSFYPPELLLRFLRNGLAAGTGQGDFGPNSDGSFHASSSLTVKSGDEHHYSCIVQHAGLAQPLRVELESPAESSHHHHHHCRNDTCG

SEQ ID NO: 94 - RNA, 25 nt, synthetic construct
  source 1..25: mol_type = other RNA; note = PCR forward primer for EC_m8
accaggattcttggtactgggagaa

SEQ ID NO: 95 - DNA, 25 bp, synthetic construct
  source 1..25: mol_type = other DNA; note = PCR reverse primer for EC_m8
caagaatcctggtcttcccaaaccc

SEQ ID NO: 96 - DNA, 25 bp, synthetic construct
  source 1..25: mol_type = other DNA; note = PCR forward primer for EC_m9
aggaagaactgttcctggaagcctt

SEQ ID NO: 97 - DNA, 25 bp, synthetic construct
  source 1..25: mol_type = other DNA; note = PCR reverse primer for EC_m9
aacagttcttccttgatgcgcagat

SEQ ID NO: 98 - DNA, 25 bp, synthetic construct
  source 1..25: mol_type = other DNA; note = PCR forward primer for EC_m10
ctgcggataaagaactgacgttcct

SEQ ID NO: 99 - DNA, 25 bp, synthetic construct
  source 1..25: mol_type = other DNA; note = PCR reverse primer for EC_m10
tctttatccgcagccttatcttgct

SEQ ID NO: 100 - DNA, 1296 bp, synthetic construct
  source 1..1296: mol_type = other DNA; note = OmpA-FcRn(B2M-GS-EC_m10)-6HC DNA
atgaaaaagacagctatcgcgattgcagtggcactggctggtttcgctaccgtagcgcaggccattcaacgtacgccaaaaatccaagtatactcacgccatccggcagagaacggtaagtctaacttcctgaattgctacgtgtctggtttccacccgtccgacatcgaagttgacctcctcaaaaacggcgaacgtatcgaaaaagttgagcactctgacctcagcttcagcaaggactggtccttctacctgctctactacacggaattcaccccgaccgagaaggatgaatacgcctgccgtgttaatcacgttaccctgtctcagccgaaaattgtgaagtgggaccgcgatatgggtggtggtggctctggcggtggtggctctggcggtggcggttccggcggcggtggtagtggtggcggcggtagcgcggaaagccatctctccctgctgtatcatctgactgcggttagctctccggcaccaggtaccccagccttctgggtctctggttggctgggtccgcagcaatacctctcttataacagcctgcgcggtgaagcagaaccacgcggtgcgtgggtttgggaagaccaggattcttggtactgggagaaagagacgaccgatctgcgcatcaaggaagaactgttcctggaagccttcaaagcgctgggcggtaaaggtccatatactctccaaggcctgctgggctgtgaactcggtcctgacaacacctctgttccgacggccaaattcgcactgaacggtgaggagtttatgaattttgacctgaaacagggcacctggggcggcgattggccagaggcgctcgctatctcccaacgctggcagcagcaagataaggctgcggataaagaactgacgttcctcctgttttcttgcccgcaccgtctccgtgaacatctcgaacttggtcgtggtgacctcgaatggaaggagcctccgtctatgcgcctgaaagcgcgtccgtcttccccggggttttctgtactcacttgttccgccttctccttttaccctccagaactcctgctgcgcttcctgcgcaatggcctcgctgcgggtacgggtcagggtgatttcggcccgaattctgacggctctttccacgcgtcttctagcctgacggtgaaatctggcgacgaacatcactacagctgcatcgtgcagcacgctggtctcgcgcaaccgctccgcgttgagctcgaatcccctgccgaatcctctcatcatcatcatcatcactgccgcaacgatacctgcgga

SEQ ID NO: 101 - protein, 220 aa, synthetic construct
PCPAPELLGGPSVFLFPPKPKDTLMISRTPEVTCVVVDVSHEDPEVKFNWYVDGVEVHNAKTKPREEQYNSTYRVVSVLTVLHQDWLNGKEYKCKVSNKALPAPIEKTISKAKGQPREPQVYTLPPSRDELTKNQVSLTCLVKGFYPSDIAVEWESNGQPENNYKTTPPVLDSDGSFFLYSKLTVDKSRWQQGNVFSCSVMHEALHNHYTQKSLSLSPGK

SEQ ID NO: 102 - protein, 220 aa, synthetic construct
PCPAPELLGGPSVFLFPPKPKDTLMISRTPEVTCVVVDVSHEDPEVKFNWYVDGVEVHNAKTKPREEQYNSTYRVVSVLTVLHQDWLNGKEYKCKVSNKALPAPIEKTISKAKGQPREPQVYTLPPSREEMTKNQVSLTCLVKGFYPSDIAVEWESNGQPENNYKTTPPVLDSDGSFFLYSKLTVDKSRWQQGNVFSCSVMHEALHNHYTQKSLSLSPGK

SEQ ID NO: 103 - protein, 220 aa, synthetic construct; identical to SEQ ID NO: 102

SEQ ID NO: 104 - protein, 220 aa, synthetic construct; identical to SEQ ID NO: 102

SEQ ID NO: 105 - protein, 220 aa, synthetic construct; identical to SEQ ID NO: 102

SEQ ID NO: 106 - protein, 219 aa, synthetic construct
PCPAPELLGGPSVFLFPPKPKDTLMISRTPEVTCVVVDVSHEDPEVKFNWYVDGVEVHNAKTKPREEQYNSTYRVVSVLTVLHQDWLNGKEYKCKVSNKALPAPIEKTISKAKGQPREPQVYTLPPSREEMTKNQVSLTCLVKGFYPSDIAVEWESNGQPENNYKTTPPVLDSDGSFFLYSKLTVDKSRWQQGNVFSCSVMHEALHNHYTQKSLSLSPG

SEQ ID NO: 107 - protein, 219 aa, synthetic construct
PCPAPELLGGPSVFLFPPKPKDTLMISRTPEVTCVVVDVSHEDPEVKFNWYVDGVEVHNAKTKPREEQYNSTYRVVSVLTVLHQDWLNGKEYKCKVSNKALPAPIEKTISKAKGQPREPQVYTLPPSRDELTKNQVSLTCLVKGFYPSDIAVEWESNGQPENNYKTTPPVLDSDGSFFLYSKLTVDKSRWQQGNVFSCSVMHEALHNHYTQKSLSLSPG

SEQ ID NO: 108 - protein, 220 aa, synthetic construct; identical to SEQ ID NO: 101

SEQ ID NO: 109 - protein, 219 aa, synthetic construct; identical to SEQ ID NO: 107

SEQ ID NO: 110 - protein, 219 aa, synthetic construct
PCPAPPVAGPSVFLFPPKPKDTLMISRTPEVTCVVVDVSHEDPEVQFNWYVDGVEVHNAKTKPREEQFNSTFRVVSVLTVVHQDWLNGKEYKCKVSNKGLPAPIEKTISKTKGQPREPQVYTLPPSREEMTKNQVSLTCLVKGFYPSDIAVEWESNGQPENNYKTTPPMLDSDGSFFLYSKLTVDKSRWQQGNVFSCSVMHEALHNHYTQKSLSLSPGK

SEQ ID NO: 111 - protein, 220 aa, synthetic construct; identical to SEQ ID NO: 101

SEQ ID NO: 112 - protein, 219 aa, synthetic construct
PCPAPEAAGGPSVFLFPPKPKDTLMISRTPEVTCVVVDVSQEDPEVQFNWYVDGVEVHNAKTKPREEQFNSTYRVVSVLTVLHQDWLNGKEYKCKVSNKGLPSSIEKTISKAKGQPREPQVYTLPPSQEEMTKNQVSLTCLVKGFYPSDIAVEWESNGQPENNYKTTPPVLDSDGSFFLYSRLTVDKSRWQEGNVFSCSVMHEALHNHYTQKSLSLSLG

SEQ ID NO: 113 - protein, 219 aa, synthetic construct; identical to SEQ ID NO: 107

SEQ ID NO: 114 - protein, 219 aa, synthetic construct; identical to SEQ ID NO: 112

SEQ ID NO: 115 - protein, 220 aa, synthetic construct
PSPAPELLGGSSVFLFPPKPKDTLMISRTPEVTCVVVDVSHEDPEVKFNWYVDGVEVHNAKTKPREEQYNSTYRVVSVLTVLHQDWLNGKEYKCKVSNKALPAPIEKTISKAKGQPREPQVYTLPPSRDELTKNQVSLTCLVKGFYPSDIAVEWESNGQPENNYKTTPPVLDSDGSFFLYSKLTVDKSRWQQGNVFSCSVMHEALHNHYTQKSLSLSPGK

SEQ ID NO: 116 - protein, 220 aa, synthetic construct
PCPAPELLGGPSVFLFPPKPKDTLMISRTPEVTCVVVDVSHEDPEVKFNWYVDGVEVHNAKTKPREEQYNSTYRVVSVLTVLHQDWLNGKEYKCKVSNKALPAPIEKTISKAKGQPREPQVYTLPPSRDELTKNQVSLTCLVKGFYPSDIAVEWESNGQPENNYKTTPPVLDSDGSFFLYSKLTVDKSRWQQGNVFSCSVMHEALHNHYTQKSLSLSPEL

SEQ ID NO: 117 - protein, 218 aa, synthetic construct
PCPAPPVAGPSVFLFPPKPKDTLMISRTPEVTCVVVDVSQEDPEVQFNWYVDGVEVHNAKTKPREEQFNSTYRVVSVLTVLHQDWLNGKEYKCKVSNKGLPSSIEKTISKAKGQPREPQVYTLPPSQEEMTKNQVSLTCLVKGFYPSDIAVEWESNGQPENNYKTTPPVLDSDGSFFLYSRLTVDKSRWQEGNVFSCSVLHEALHSHYTQKSLSLSLG

SEQ ID NO: 118 - protein, 437 aa, synthetic construct
MKIKTGARILALSALTTMMFSASALAKIEEAMGIQRTPKIQVYSRHPAENGKSNFLNCYVSGFHPSDIEVDLLKNGERIEKVEHSDLSFSKDWSFYLLYYTEFTPTEKDEYACRVNHVTLSQPKIVKWDRDMGGGGSGGGGSGGGGSGGGGSGGGGSAESHLSLLYHLTAVSSPAPGTPAFWVSGWLGPQQYLSYNSLRGEAEPCGAWVWENQVSWYWEKETTDLRIKEKLFLEAFKALGGKGPYTLQGLLGCELGPDNTSVPTAKFALNGEEFMNFDLKQGTWGGDWPEALAISQRWQQQDKAANKELTFLLFSCPHRLREHLERGRGNLEWKEPPSMRLKARPSSPGFSVLTCSAFSFYPPELQLRFLRNGLAAGTGQGDFGPNSDGSFHASSSLTVKSGDEHHYCCIVQHAGLAQPLRVELESPAKSSHHHHHH

SEQ ID NO: 119 - DNA, 1314 bp, synthetic construct
  source 1..1314: mol_type = other DNA
atgaaaataaaaacaggtgcacgcatcctcgcattatccgcattaacgacgatgatgttttccgcctcggctctcgccaaaatcgaagaagccatgggcattcaacgtacgccaaaaatccaagtttactctcgccatccggcagagaacggtaagtctaacttcctgaattgctacgtgtctggtttccacccgtccgacatcgaagttgacctcctcaaaaacggcgaacgtatcgaaaaagttgagcactctgacctcagcttcagcaaggactggtccttctacctgctctactacacggaattcaccccgaccgagaaggatgaatacgcctgccgtgttaatcacgttaccctgtctcagccgaaaattgtgaagtgggaccgcgatatgggtggtggtggctctggcggtggcggctctggcggtggcggttccggcggcggtggtagcggtggcggcggtagcgcggaaagccatctctccctgctgtatcatctgactgcggttagctctccggcaccaggtaccccagccttctgggtctctggttggctgggtccgcagcaatacctctcttataacagcctgcgcggtgaagcagaaccatgcggtgcgtgggtttgggaaaaccaggtttcttggtactgggagaaagagacgaccgatctgcgcatcaaggaaaaactgttcctggaagccttcaaagcgctgggcggtaaaggtccatatactctccaaggcctgctgggctgtgaactcggtcctgacaacacctctgttccgacggccaaattcgcactgaacggtgaggagtttatgaattttgacctgaaacagggcacctggggtggcgattggccagaggcgctcgctatctcccaacgctggcagcagcaagataaggcagcgaacaaagaactgacgttcctcctgttttcttgcccgcaccgtctccgtgaacatctcgaacgtggtcgtggtaacctcgaatggaaggagcctccgtctatgcgtctgaaagcgcgtccgtcttccccgggtttttctgtactcacttgttccgccttctccttttaccctccagaactccagctgcgcttcctgcgcaatggcctcgctgcgggtacgggtcagggtgatttcggcccgaattctgacggctctttccacgcgtcttctagcctgacggtgaaatctggcgacgaacatcactactgctgcatcgtgcagcacgcgggtctcgcgcaaccgctccgcgttgagctcgaatcccctgccaaatcttctcatcatcatcatcatcattaa